European Patent Application EP 4 212 168 A1, published July 19, 2023. Title: A Novel Composition for Preventing or Treating Staphylococcus aureus infectious diseases. Applicant: Clips. The sequence listing filed with the application follows.

SEQUENCE LISTING (54 sequences)

SEQ ID NO: 1 - DNA, 29 bp, Artificial Sequence
  Vector-pET28a-F primer
catggtatatctccttcttaaagttaaac

SEQ ID NO: 2 - DNA, 25 bp, Artificial Sequence
  Vector-pET28a-R primer
caccaccaccaccaccactgagatc

SEQ ID NO: 3 - DNA, 49 bp, Artificial Sequence
  pET28a-6 His-LukS-R primer
gtggtggtggtggtgattatgtcctttcactttaatttcatgagttttc

SEQ ID NO: 4 - DNA, 54 bp, Artificial Sequence
  pET28a-6 His-LukS-F primer
ctttaagaaggagatataccatggataacaatattgagaatattggtgatggcg

SEQ ID NO: 5 - DNA, 29 bp, Artificial Sequence
  pET28a-6 His-LukST244A-R primer
catggtatatctccttcttaaagttaaac

SEQ ID NO: 6 - DNA, 37 bp, Artificial Sequence
  pET28a-6 His-LukST244A-F primer
ctattgccatagtgtgctgttcttctagtagcatgag

SEQ ID NO: 7 - DNA, 44 bp, Artificial Sequence
  pET28a-6 His-LukF-R primer
gtggtggtggtggtggctcataggatttttttccttagattgag

SEQ ID NO: 8 - DNA, 50 bp, Artificial Sequence
  pET28a-6 His-LukF-F primer
ctttaagaaggagatataccatggctcaacatatcacacctgtaagtgag

SEQ ID NO: 9 - DNA, 45 bp, Artificial Sequence
  pET28a-6 His-HlgA-R primer
gtggtggtggtggtgcttaggtgtgatgcttttaatttttacttc

SEQ ID NO: 10 - DNA, 55 bp, Artificial Sequence
  pET28a-6 His-HlgA-F primer
ctttaagaaggagatataccatggaaaataagatagaagatatcggccaaggtgc

SEQ ID NO: 11 - DNA, 42 bp, Artificial Sequence
  pET28a-6 His-HlgC-R primer
gtggtggtggtggtgattctgtcctttcaccttgatttcatg

SEQ ID NO: 12 - DNA, 51 bp, Artificial Sequence
  pET28a-6 His-HlgC-F primer
ctttaagaaggagatataccatgctaacgatactgaagacatcggtaaagg

SEQ ID NO: 13 - DNA, 48 bp, Artificial Sequence
  pET28a-6 His-LukE-R primer
gtggtggtggtggtgttatgtcctttcactttaatttcgtgtgttttc

SEQ ID NO: 14 - DNA, 57 bp, Artificial Sequence
  pET28a-6 His-LukE-F primer
ctttaagaaggagatataccatgaatactaatattgaaaatattggtgatggtgctg

SEQ ID NO: 15 - DNA, 44 bp, Artificial Sequence
  pET28a-6 His-LukD-R primer
gtggtggtggtggtgtactccaggattagtttctttagaatccg

SEQ ID NO: 16 - DNA, 48 bp, Artificial Sequence
  pET28a-6 His-LukD-F primer
ctttaagaaggagatataccatggctcaacatatcacacctgtaagcg

SEQ ID NO: 17 - DNA, 46 bp, Artificial Sequence
  pET28a-6 His-Hla-R primer
cagtggtggtggtggtggtgatttgtcatttcttctttttcccaat

SEQ ID NO: 18 - DNA, 48 bp, Artificial Sequence
  pET28a-6 His-Hla-F primer
aagaaggagatataccatggcagattctgatattaatattaaaaccgg

SEQ ID NO: 19 - DNA, 37 bp, Artificial Sequence
  pET28a-6 His-HlaH35L-R primer
gaagaacgatctatccatttatctttagtattggtac

SEQ ID NO: 20 - DNA, 46 bp, Artificial Sequence
  pET28a-6 His-HlaH35L-F primer
gataaagaaaatggcatgctcaaaaaagtattttatagttttatcg

SEQ ID NO: 21 - DNA, 22 bp, Artificial Sequence
  Vector-pET28a-R primer
gtgatgatgatgatgatggctg

SEQ ID NO: 22 - DNA, 25 bp, Artificial Sequence
  Vector-pET28a-F primer
caccaccaccaccaccactgagatc

SEQ ID NO: 23 - DNA, 54 bp, Artificial Sequence
  pET28a-6 His-hlgB-R primer
ttgttagcagccggatctcatttattgttttcagtttcttttgtatctaacaat

SEQ ID NO: 24 - DNA, 47 bp, Artificial Sequence
  pET28a-6 His-hlgB-F primer
atgggcagcagccatcatcatcatcatcacgaaggtaaaataacacc

SEQ ID NO: 25 - DNA, 57 bp, Artificial Sequence
  pET28a-6 His-LukA-R primer
atgggcagcagccatcatcatcatcatcacaattcagctcataaagactctcaagac

SEQ ID NO: 26 - DNA, 53 bp, Artificial Sequence
  pET28a-6 His-LukA-F primer
tagtaatccgccctttcaatattatccttctttataaggtttattgtcatcag

SEQ ID NO: 27 - DNA, 56 bp, Artificial Sequence
  pET28a-6 His-LukB-R primer
cagtggtggtggtggtggtgttatttcttttcattatcattaagtacttttacaaa

SEQ ID NO: 28 - DNA, 53 bp, Artificial Sequence
  pET28a-6 His-LukB-F primer
tattgaaagggcggattactaatgaagattaattctgaaatcaaacaagtttc

SEQ ID NO: 29 - DNA, 53 bp, Artificial Sequence
  pET28a-6 His-LukAE323A-F primer
tagtaatccgccctttcaatattatcctgctttataaggtttattgtcatcag

SEQ ID NO: 30 - DNA, 57 bp, Artificial Sequence; identical to SEQ ID NO: 25
  pET28a-6 His-LukAE323A-R primer

SEQ ID NO: 31 - DNA, 47 bp, Artificial Sequence
  clfA-F primer
ttgttagcagccggatctcatgaattagaatcgctgccagaatctga

SEQ ID NO: 32 - DNA, 55 bp, Artificial Sequence
  clfA-R primer
atgggcagcagccatcatcatcatcatcacgcatttagtttagcggcagtagctg

SEQ ID NO: 33 - DNA, 39 bp, Artificial Sequence
  clfB-F primer
ttgttagcagccggatctcattctgggtcaaccggcggc

SEQ ID NO: 34 - DNA, 53 bp, Artificial Sequence
  clfB-R primer
atgggcagcagccatcatcatcatcatcacgttgctgaaccggtagtaaatgc

SEQ ID NO: 35 - DNA, 51 bp, Artificial Sequence
  sdrC-F primer
ctttaagaaggagatataccatgagaactttaaatcgcatggcagtgaata

SEQ ID NO: 36 - DNA, 47 bp, Artificial Sequence
  sdrC-R primer
cagtggtggtggtggtggtgtgtatcttcccatacatagtcacctag

SEQ ID NO: 37 - DNA, 51 bp, Artificial Sequence
  sdrD-F primer
ctttaagaaggagatataccatggcacctaaacgtttgaatacaagaatgc

SEQ ID NO: 38 - DNA, 43 bp, Artificial Sequence
  sdrD-R primer
cagtggtggtggtggtggtgatatacttcttgaccagctccgc

SEQ ID NO: 39 - DNA, 54 bp, Artificial Sequence
  sdrE-F primer
ttgttagcagccggatctcaaattttgtataacttttcttcaggtttaacagta

SEQ ID NO: 40 - DNA, 55 bp, Artificial Sequence
  sdrE-R primer
atgggcagcagccatcatcatcatcatcacgtaaacgcaaaaatgcgctttgcag

SEQ ID NO: 41 - DNA, 49 bp, Artificial Sequence
  fnbpA-F primer
ctttaagaaggagatataccatggtagcggaagctaaggaagctagtaa

SEQ ID NO: 42 - DNA, 46 bp, Artificial Sequence
  fnbpA-R primer
cagtggtggtggtggtggtgagctgtgtggtaatcaatgtcaagag

SEQ ID NO: 43 - DNA, 46 bp, Artificial Sequence
  fnbpB-F primer
taagaaggagatataccatgatgaaaagatcaactgacgttacagc

SEQ ID NO: 44 - DNA, 41 bp, Artificial Sequence
  fnbpB-R primer
cagtggtggtggtggtggtgcactggcggctctgatttaaa

SEQ ID NO: 45 - DNA, 26 bp, Artificial Sequence
  pET28a-C-fragment1-F primer
gcatcctctctcgtttcatcggtatc

SEQ ID NO: 46 - DNA, 25 bp, Artificial Sequence
  pET28a-C-fragment1-R primer
caccaccaccaccaccactgagatc

SEQ ID NO: 47 - DNA, 29 bp, Artificial Sequence
  pET28a-C-fragment2-F primer
catggtatatctccttcttaaagttaaac

SEQ ID NO: 48 - DNA, 26 bp, Artificial Sequence
  pET28a-C-fragment2-R primer
gaaacgagagaggatgctcacgatac

SEQ ID NO: 49 - DNA, 26 bp, Artificial Sequence
  pET28a-N-fragment1-F primer
gcatcctctctcgtttcatcggtatc

SEQ ID NO: 50 - DNA, 23 bp, Artificial Sequence
  pET28a-N-fragment1-R primer
tgagatccggctgctaacaaagc

SEQ ID NO: 51 - DNA, 23 bp, Artificial Sequence
  pET28a-N-fragment2-F primer
gtgatgatgatgatgatggctgc

SEQ ID NO: 52 - DNA, 26 bp, Artificial Sequence
  pET28a-N-fragment2-R primer
gaaacgagagaggatgctcacgatac

SEQ ID NO: 53 - DNA, 23 bp, Artificial Sequence
  T7 promoter
aaattaatacgactcactatagg

SEQ ID NO: 54 - DNA, 21 bp, Artificial Sequence
  T7 terminator
atgctagttattgctcagcgg